European Patent Application EP 4 129 333 A1, published February 8, 2023. Title: Medicament for killing tumor cells. Applicant: PhotoQ3 Inc. The sequence listing filed with the application follows.

SEQUENCE LISTING (3 sequences)

SEQ ID NO: 1 - protein, 12 aa, Artificial Sequence
  Description of Artificial Sequence: artificial peptide
YHWYGYTPQNVI

SEQ ID NO: 2 - protein, 6 aa, Artificial Sequence
  Description of Artificial Sequence: artificial peptide
LARLLT

SEQ ID NO: 3 - protein, 12 aa, Artificial Sequence
  Description of Artificial Sequence: artificial peptide
YHWYGYTPENVI